European Patent Application EP 4 431 529 A1, published September 18, 2024. Title: 一种抗IL-17/VEGF双功能融合蛋白及其用途. Applicant: 三生国健药业（上海）股份有限公司. The sequence listing filed with the application follows.

SEQUENCE LISTING (34 sequences)

SEQ ID NO: 1 - protein, 214 aa, synthetic construct
DIQMTQSPSSLSASVGDRVTITCKASDHINNWLAWYQQKPGKAPKLLISGATSLETGVPSRFSGSGSGTDYTLTISSLQPEDFATYYCQQYWSTPFTFGSGTKLEIKRTVAAPSVFIFPPSDEQLKSGTASVVCLLNNFYPREAKVQWKVDNALQSGNSQESVTEQDSKDSTYSLSSTLTLSKADYEKHKVYACEVTHQGLSSPVTKSFNRGEC

SEQ ID NO: 2 - protein, 553 aa, synthetic construct
EVQLVESGGGLVQPGGSLRLSCAASGFTFSSFDMSWGRQAPGKRLEWVAFMSSGGSTYYPDSVKGRFTISRDNSKNTLYLQMNSLRAEDTAVYYCARGERYGSYWGQGTLVTVSSASTKGPSVFPLAPSSKSTSGGTAALGCLVKDYFPEPVTVSWNSGALTSGVHTFPAVLQSSGLYSLSSVVTVPSSSLGTQTYICNVNHKPSNTKVDKKVEPKSCDKTHTCPPCPAPELLGGPSVFLFPPKPKDTLMISRTPEVTCVVVDVSHEDPEVKFNWYVDGVEVHNAKTKPREEQYNSTYRVVSVLTVLHQDWLNGKEYKCKVSNKALPAPIEKTISKAKGQPREPQVYTLPPSREEMTKNQVSLTCLVKGFYPSDIAVEWESNGQPENNYKTTPPVLDSDGSFFLYSKLTVDKSRWQQGNVFSCSVMHEALHNHYTQKSLSLSPGAGGGGSGGGGSDTGRPFVEMYSEIPEIIHMTEGRELVIPCRVTSPNITVTLKKFPLDTLIPDGKRIIWDSRKGFIISNATYKEIGLLTCEATVNGHLYKTNYLTHRQTN

SEQ ID NO: 3 - protein, 563 aa, synthetic construct
DTGRPFVEMYSEIPEIIHMTEGRELVIPCRVTSPNITVTLKKFPLDTLIPDGKRIIWDSRKGFIISNATYKEIGLLTCEATVNGHLYKTNYLTHRQTNGGGGSGGGGSGGGGSGGGGSEVQLVESGGGLVQPGGSLRLSCAASGFTFSSFDMSWGRQAPGKRLEWVAFMSSGGSTYYPDSVKGRFTISRDNSKNTLYLQMNSLRAEDTAVYYCARGERYGSYWGQGTLVTVSSASTKGPSVFPLAPSSKSTSGGTAALGCLVKDYFPEPVTVSWNSGALTSGVHTFPAVLQSSGLYSLSSVVTVPSSSLGTQTYICNVNHKPSNTKVDKKVEPKSCDKTHTCPPCPAPELLGGPSVFLFPPKPKDTLMISRTPEVTCVVVDVSHEDPEVKFNWYVDGVEVHNAKTKPREEQYNSTYRVVSVLTVLHQDWLNGKEYKCKVSNKALPAPIEKTISKAKGQPREPQVYTLPPSREEMTKNQVSLTCLVKGFYPSDIAVEWESNGQPENNYKTTPPVLDSDGSFFLYSKLTVDKSRWQQGNVFSCSVMHEALHNHYTQKSLSLSPGK

SEQ ID NO: 4 - protein, 445 aa, synthetic construct
EVQLVESGGGLVQPGGSLRLSCAASGFTFSSFDMSWGRQAPGKRLEWVAFMSSGGSTYYPDSVKGRFTISRDNSKNTLYLQMNSLRAEDTAVYYCARGERYGSYWGQGTLVTVSSASTKGPSVFPLAPSSKSTSGGTAALGCLVKDYFPEPVTVSWNSGALTSGVHTFPAVLQSSGLYSLSSVVTVPSSSLGTQTYICNVNHKPSNTKVDKKVEPKSCDKTHTCPPCPAPELLGGPSVFLFPPKPKDTLMISRTPEVTCVVVDVSHEDPEVKFNWYVDGVEVHNAKTKPREEQYNSTYRVVSVLTVLHQDWLNGKEYKCKVSNKALPAPIEKTISKAKGQPREPQVYTLPPSREEMTKNQVSLTCLVKGFYPSDIAVEWESNGQPENNYKTTPPVLDSDGSFFLYSKLTVDKSRWQQGNVFSCSVMHEALHNHYTQKSLSLSPGK

SEQ ID NO: 5 - protein, 322 aa, synthetic construct
DIQMTQSPSSLSASVGDRVTITCKASDHINNWLAWYQQKPGKAPKLLISGATSLETGVPSRFSGSGSGTDYTLTISSLQPEDFATYYCQQYWSTPFTFGSGTKLEIKRTVAAPSVFIFPPSDEQLKSGTASVVCLLNNFYPREAKVQWKVDNALQSGNSQESVTEQDSKDSTYSLSSTLTLSKADYEKHKVYACEVTHQGLSSPVTKSFNRGECGGGGSGGGGSDTGRPFVEMYSEIPEIIHMTEGRELVIPCRVTSPNITVTLKKFPLDTLIPDGKRIIWDSRKGFIISNATYKEIGLLTCEATVNGHLYKTNYLTHRQTN

SEQ ID NO: 6 - protein, 332 aa, synthetic construct
DTGRPFVEMYSEIPEIIHMTEGRELVIPCRVTSPNITVTLKKFPLDTLIPDGKRIIWDSRKGFIISNATYKEIGLLTCEATVNGHLYKTNYLTHRQTNGGGGSGGGGSGGGGSGGGGSDIQMTQSPSSLSASVGDRVTITCKASDHINNWLAWYQQKPGKAPKLLISGATSLETGVPSRFSGSGSGTDYTLTISSLQPEDFATYYCQQYWSTPFTFGSGTKLEIKRTVAAPSVFIFPPSDEQLKSGTASVVCLLNNFYPREAKVQWKVDNALQSGNSQESVTEQDSKDSTYSLSSTLTLSKADYEKHKVYACEVTHQGLSSPVTKSFNRGEC

SEQ ID NO: 7 - protein, 553 aa, synthetic construct
EVQLVESGGGLVQPGGSLRLSCAASGFTFSSFDMSWGRQAPGKRLEWVAFMSSGGSTYYPDSVKGRFTISRDNSKNTLYLQMNSLRAEDTAVYYCARGERYGSYWGQGTLVTVSSASTKGPSVFPLAPSSKSTSGGTAALGCLVKDYFPEPVTVSWNSGALTSGVHTFPAVLQSSGLYSLSSVVTVPSSSLGTQTYICNVNHKPSNTKVDKKVEPKSCDKTHTCPPCPAPELLGGPSVFLFPPKPKDTLMISRTPEVTCVVVDVSHEDPEVKFNWYVDGVEVHNAKTKPREEQYNSTYRVVSVLTVLHQDWLNGKEYKCKVSNKALPAPIEKTISKAKGQPREPQVYTLPPSREEMTKNQVSLTCLVKGFYPSDIAVEWESNGQPENNYKTTPPVLDSDGSFFLYSKLTVDKSRWQQGNVFSCSVMHEALHNHYTQKSLSLSPGAGGGGSGGGGSDTGRPFVEAYSEIPEIIHMTEGRELVIPCRVTSPNITVTLKKFPLDTLIPDGKRIIWDSRKGFIISNATYKEIGLLTCEATVNGHLYKTNYLTHRQTN

SEQ ID NO: 8 - protein, 553 aa, synthetic construct
EVQLVESGGGLVQPGGSLRLSCAASGFTFSSFDMSWGRQAPGKRLEWVAFMSSGGSTYYPDSVKGRFTISRDNSKNTLYLQMNSLRAEDTAVYYCARGERYGSYWGQGTLVTVSSASTKGPSVFPLAPSSKSTSGGTAALGCLVKDYFPEPVTVSWNSGALTSGVHTFPAVLQSSGLYSLSSVVTVPSSSLGTQTYICNVNHKPSNTKVDKKVEPKSCDKTHTCPPCPAPELLGGPSVFLFPPKPKDTLMISRTPEVTCVVVDVSHEDPEVKFNWYVDGVEVHNAKTKPREEQYNSTYRVVSVLTVLHQDWLNGKEYKCKVSNKALPAPIEKTISKAKGQPREPQVYTLPPSREEMTKNQVSLTCLVKGFYPSDIAVEWESNGQPENNYKTTPPVLDSDGSFFLYSKLTVDKSRWQQGNVFSCSVMHEALHNHYTQKSLSLSPGAGGGGSGGGGSDTGRPFVEPYSEIPEIIHMTEGRELVIPCRVTSPNITVTLKKFPLDTLIPDGKRIIWDSRKGFIISNATYKEIGLLTCEATVNGHLYKTNYLTHRQTN

SEQ ID NO: 9 - protein, 553 aa, synthetic construct
EVQLVESGGGLVQPGGSLRLSCAASGFTFSSFDMSWGRQAPGKRLEWVAFMSSGGSTYYPDSVKGRFTISRDNSKNTLYLQMNSLRAEDTAVYYCARGERYGSYWGQGTLVTVSSASTKGPSVFPLAPSSKSTSGGTAALGCLVKDYFPEPVTVSWNSGALTSGVHTFPAVLQSSGLYSLSSVVTVPSSSLGTQTYICNVNHKPSNTKVDKKVEPKSCDKTHTCPPCPAPELLGGPSVFLFPPKPKDTLMISRTPEVTCVVVDVSHEDPEVKFNWYVDGVEVHNAKTKPREEQYNSTYRVVSVLTVLHQDWLNGKEYKCKVSNKALPAPIEKTISKAKGQPREPQVYTLPPSREEMTKNQVSLTCLVKGFYPSDIAVEWESNGQPENNYKTTPPVLDSDGSFFLYSKLTVDKSRWQQGNVFSCSVMHEALHNHYTQKSLSLSPGAGGGGSGGGGSDTGRPFVETYSEIPEIIHMTEGRELVIPCRVTSPNITVTLKKFPLDTLIPDGKRIIWDSRKGFIISNATYKEIGLLTCEATVNGHLYKTNYLTHRQTN

SEQ ID NO: 10 - protein, 553 aa, synthetic construct
EVQLVESGGGLVQPGGSLRLSCAASGFTFSSFDMSWGRQAPGKRLEWVAFMSSGGSTYYPDSVKGRFTISRDNSKNTLYLQMNSLRAEDTAVYYCARGERYGSYWGQGTLVTVSSASTKGPSVFPLAPSSKSTSGGTAALGCLVKDYFPEPVTVSWNSGALTSGVHTFPAVLQSSGLYSLSSVVTVPSSSLGTQTYICNVNHKPSNTKVDKKVEPKSCDKTHTCPPCPAPELLGGPSVFLFPPKPKDTLMISRTPEVTCVVVDVSHEDPEVKFNWYVDGVEVHNAKTKPREEQYNSTYRVVSVLTVLHQDWLNGKEYKCKVSNKALPAPIEKTISKAKGQPREPQVYTLPPSREEMTKNQVSLTCLVKGFYPSDIAVEWESNGQPENNYKTTPPVLDSDGSFFLYSKLTVDKSRWQQGNVFSCSVMHEALHNHYTQKSLSLSPGAGGGGSGGGGSDTGRPFVEAASEIPEIIHMTEGRELVIPCRVTSPNITVTLKKFPLDTLIPDGKRIIWDSRKGFIISNATYKEIGLLTCEATVNGHLYKTNYLTHRQTN

SEQ ID NO: 11 - protein, 337 aa, synthetic construct
DKTHTCPPCPAPELLGGPSVFLFPPKPKDTLMISRTPEVTCVVVDVSHEDPEVKFNWYVDGVEVHNAKTKPREEQYNSTYRVVSVLTVLHQDWLNGKEYKCKVSNKALPAPIEKTISKAKGQPREPQVYTLPPSREEMTKNQVSLTCLVKGFYPSDIAVEWESNGQPENNYKTTPPVLDSDGSFFLYSKLTVDKSRWQQGNVFSCSVMHEALHNHYTQKSLSLSPGKGGGGSGGGGSDTGRPFVEMYSEIPEIIHMTEGRELVIPCRVTSPNITVTLKKFPLDTLIPDGKRIIWDSRKGFIISNATYKEIGLLTCEATVNGHLYKTNYLTHRQTNTI

SEQ ID NO: 12 - protein, 453 aa, synthetic construct
EVQLVESGGGLVQPGGSLRLSCAASGYTFTNYGMNWVRQAPGKGLEWVGWINTYTGEPTYAADFKRRFTFSLDTSKSTAYLQMNSLRAEDTAVYYCAKYPHYYGSSHWYFDVWGQGTLVTVSSASTKGPSVFPLAPSSKSTSGGTAALGCLVKDYFPEPVTVSWNSGALTSGVHTFPAVLQSSGLYSLSSVVTVPSSSLGTQTYICNVNHKPSNTKVDKKVEPKSCDKTHTCPPCPAPELLGGPSVFLFPPKPKDTLMISRTPEVTCVVVDVSHEDPEVKFNWYVDGVEVHNAKTKPREEQYNSTYRVVSVLTVLHQDWLNGKEYKCKVSNKALPAPIEKTISKAKGQPREPQVYTLPPSREEMTKNQVSLTCLVKGFYPSDIAVEWESNGQPENNYKTTPPVLDSDGSFFLYSKLTVDKSRWQQGNVFSCSVMHEALHNHYTQKSLSLSPGK

SEQ ID NO: 13 - protein, 214 aa, synthetic construct
DIQMTQSPSSLSASVGDRVTITCSASQDISNYLNWYQQKPGKAPKVLIYFTSSLHSGVPSRFSGSGSGTDFTLTISSLQPEDFATYYCQQYSTVPWTFGQGTKVEIKRTVAAPSVFIFPPSDEQLKSGTASVVCLLNNFYPREAKVQWKVDNALQSGNSQESVTEQDSKDSTYSLSSTLTLSKADYEKHKVYACEVTHQGLSSPVTKSFNRGEC

SEQ ID NO: 14 - protein, 5 aa, synthetic construct
SFDMS

SEQ ID NO: 15 - protein, 16 aa, synthetic construct
FMSSGGSTYYPDSVKG

SEQ ID NO: 16 - protein, 7 aa, synthetic construct
GERYGSY

SEQ ID NO: 17 - protein, 11 aa, synthetic construct
KASDHINNWLA

SEQ ID NO: 18 - protein, 7 aa, synthetic construct
GATSLET

SEQ ID NO: 19 - protein, 9 aa, synthetic construct
QQYWSTPFT

SEQ ID NO: 20 - protein, 115 aa, synthetic construct
EVQLVESGGGLVQPGGSLRLSCAASGFTFSSFDMSWGRQAPGKRLEWVAFMSSGGSTYYPDSVKGRFTISRDNSKNTLYLQMNSLRAEDTAVYYCARGERYGSYWGQGTLVTVSS

SEQ ID NO: 21 - protein, 107 aa, synthetic construct
DIQMTQSPSSLSASVGDRVTITCKASDHINNWLAWYQQKPGKAPKLLISGATSLETGVPSRFSGSGSGTDYTLTISSLQPEDFATYYCQQYWSTPFTFGSGTKLEIK

SEQ ID NO: 22 - protein, 330 aa, synthetic construct
ASTKGPSVFPLAPSSKSTSGGTAALGCLVKDYFPEPVTVSWNSGALTSGVHTFPAVLQSSGLYSLSSVVTVPSSSLGTQTYICNVNHKPSNTKVDKKVEPKSCDKTHTCPPCPAPELLGGPSVFLFPPKPKDTLMISRTPEVTCVVVDVSHEDPEVKFNWYVDGVEVHNAKTKPREEQYNSTYRVVSVLTVLHQDWLNGKEYKCKVSNKALPAPIEKTISKAKGQPREPQVYTLPPSREEMTKNQVSLTCLVKGFYPSDIAVEWESNGQPENNYKTTPPVLDSDGSFFLYSKLTVDKSRWQQGNVFSCSVMHEALHNHYTQKSLSLSPGK

SEQ ID NO: 23 - protein, 107 aa, synthetic construct [sequence omitted]

SEQ ID NO: 24 - DNA, 714 bp, synthetic construct
  source 1..714: mol_type = other DNA
atggacacccgcgcccccacccagctgctgggcctgctgctgctgtggcttcccggcgcccgatgcgatattcagatgacccagagcccaagcagcctgtccgcatctgtcggagatagggtgactatcacctgcaaggcttccgaccacatcaacaattggctcgcctggtaccagcagaagcctggaaaggcccctaagttgctcatctccggcgccacatctcttgaaaccggggtgccaagtcggttttcagggagtggcagcgggactgactatacactgacaatttcctccctgcaacccgaggacttcgccacatactactgtcagcagtactggagcacaccctttactttcgggagcggcaccaaactggagattaagagaaccgtcgccgctcccagcgtcttcatcttcccccccagcgatgagcagctgaagagcggaaccgccagcgtggtgtgcctgctgaacaacttctaccccagggaggccaaggtgcaatggaaggtggacaacgccctacagagcggcaactcccaggagagcgtgaccgagcaggacagcaaggatagcacctacagcctgagcagcaccctcaccctgagcaaggccgactacgagaagcacaaggtgtacgcctgcgaggtgacccatcagggcctgagcagccctgtgaccaagagcttcaacaggggcgagtgctgataa

SEQ ID NO: 25 - DNA, 1665 bp, synthetic construct
  source 1..1665: mol_type = other DNA
gaggtgcagctcgtcgaatctggaggcggcctcgtgcagcctggggggtctcttagattgtcctgcgcagcttcaggattcactttctccagcttcgacatgagctgggggaggcaggctccagggaagaggctggagtgggtcgcctttatgtcctccggaggcagtacatactaccccgatagtgtgaaagggaggtttaccatcagccgcgacaacagcaagaacaccctgtacctgcagatgaatagcctgcgggccgaggatacagccgtctactactgtgcccggggcgagcggtacggctcctattggggccaagggacactggtgactgtgagctccgcgagcaccaagggaccttccgtgtttcccctcgcccccagctccaaaagcaccagcggcggaacagctgctctcggctgtctcgtcaaggattacttccccgagcccgtgaccgtgagctggaacagcggagccctgacaagcggcgtccacaccttccctgctgtcctacagtcctccggactgtacagcctgagcagcgtggtgacagtccctagcagctccctgggcacccagacatatatttgcaacgtgaatcacaagcccagcaacaccaaggtcgataagaaggtggagcctaagtcctgcgacaagacccacacatgtcccccctgtcccgctcctgaactgctgggaggcccttccgtgttcctgttcccccctaagcccaaggacaccctgatgatttccaggacacccgaggtgacctgtgtggtggtggacgtcagccacgaggaccccgaggtgaaattcaactggtacgtcgatggcgtggaggtgcacaacgctaagaccaagcccagggaggagcagtacaattccacctacagggtggtgtccgtgctgaccgtcctccatcaggactggctgaacggcaaagagtataagtgcaaggtgagcaacaaggccctccctgctcccatcgagaagaccatcagcaaagccaagggccagcccagggaacctcaagtctataccctgcctcccagcagggaggagatgaccaagaaccaagtgagcctcacatgcctcgtcaagggcttctatccttccgatattgccgtcgagtgggagtccaacggacagcccgagaacaactacaagacaacaccccccgtgctcgattccgatggcagcttcttcctgtactccaagctgaccgtggacaagtccagatggcaacaaggcaacgtcttcagttgcagcgtcatgcatgaggccctccacaaccactacacccagaagagcctctccctgagccctggagccggcggaggcggaagcggaggaggaggatccgatactggaaggccatttgtggagatgtacagcgagatcccagagatcattcacatgacagaaggaagggagctcgtcatcccatgcagagtgacaagccctaacatcactgtcactctcaagaagttcccactcgacacactcatcccagatggcaagagaatcatttgggacagcagaaagggcttcatcatctccaacgccacatataaggagatcggactgctcacttgcgaagctacagtcaacggccacctctataagactaactatctgactcataggcaaacaaactgataa

SEQ ID NO: 26 - DNA, 1692 bp, synthetic construct
  source 1..1692: mol_type = other DNA
gatactggaaggccatttgtggagatgtacagcgagatcccagagatcattcacatgacagaaggaagggagctcgtcatcccatgcagagtgacaagccctaacatcactgtcactctcaagaagttcccactcgacacactcatcccagatggcaagagaatcatttgggacagcagaaagggcttcatcatctccaacgccacatataaggagatcggactgctcacttgcgaagctacagtcaacggccacctctataagactaactatctgactcataggcaaacaaacggtggaggcggttcaggcggaggtggcagcggcggtggcgggtcgggagggggtggctctgaggtgcagctcgtcgaatctggaggcggcctcgtgcagcctggggggtctcttagattgtcctgcgcagcttcaggattcactttctccagcttcgacatgagctgggggaggcaggctccagggaagaggctggagtgggtcgcctttatgtcctccggaggcagtacatactaccccgatagtgtgaaagggaggtttaccatcagccgcgacaacagcaagaacaccctgtacctgcagatgaatagcctgcgggccgaggatacagccgtctactactgtgcccggggcgagcggtacggctcctattggggccaagggacactggtgactgtgagctccgcgagcaccaagggaccttccgtgtttcccctcgcccccagctccaaaagcaccagcggcggaacagctgctctcggctgtctcgtcaaggattacttccccgagcccgtgaccgtgagctggaacagcggagccctgacaagcggcgtccacaccttccctgctgtcctacagtcctccggactgtacagcctgagcagcgtggtgacagtccctagcagctccctgggcacccagacatatatttgcaacgtgaatcacaagcccagcaacaccaaggtcgataagaaggtggagcctaagtcctgcgacaagacccacacatgtcccccctgtcccgctcctgaactgctgggaggcccttccgtgttcctgttcccccctaagcccaaggacaccctgatgatttccaggacacccgaggtgacctgtgtggtggtggacgtcagccacgaggaccccgaggtgaaattcaactggtacgtcgatggcgtggaggtgcacaacgctaagaccaagcccagggaggagcagtacaattccacctacagggtggtgtccgtgctgaccgtcctccatcaggactggctgaacggcaaagagtataagtgcaaggtgagcaacaaggccctccctgctcccatcgagaagaccatcagcaaagccaagggccagcccagggaacctcaagtctataccctgcctcccagcagggaggagatgaccaagaaccaagtgagcctcacatgcctcgtcaagggcttctatccttccgatattgccgtcgagtgggagtccaacggacagcccgagaacaactacaagacaacaccccccgtgctcgattccgatggcagcttcttcctgtactccaagctgaccgtggacaagtccagatggcaacaaggcaacgtcttcagttgcagcgtcatgcatgaggccctccacaaccactacacccagaagagcctctccctgagccctggaaagtga

SEQ ID NO: 27 - DNA, 1338 bp, synthetic construct
  source 1..1338: mol_type = other DNA
gaggtgcagctcgtcgaatctggaggcggcctcgtgcagcctggggggtctcttagattgtcctgcgcagcttcaggattcactttctccagcttcgacatgagctgggggaggcaggctccagggaagaggctggagtgggtcgcctttatgtcctccggaggcagtacatactaccccgatagtgtgaaagggaggtttaccatcagccgcgacaacagcaagaacaccctgtacctgcagatgaatagcctgcgggccgaggatacagccgtctactactgtgcccggggcgagcggtacggctcctattggggccaagggacactggtgactgtgagctccgcgagcaccaagggaccttccgtgtttcccctcgcccccagctccaaaagcaccagcggcggaacagctgctctcggctgtctcgtcaaggattacttccccgagcccgtgaccgtgagctggaacagcggagccctgacaagcggcgtccacaccttccctgctgtcctacagtcctccggactgtacagcctgagcagcgtggtgacagtccctagcagctccctgggcacccagacatatatttgcaacgtgaatcacaagcccagcaacaccaaggtcgataagaaggtggagcctaagtcctgcgacaagacccacacatgtcccccctgtcccgctcctgaactgctgggaggcccttccgtgttcctgttcccccctaagcccaaggacaccctgatgatttccaggacacccgaggtgacctgtgtggtggtggacgtcagccacgaggaccccgaggtgaaattcaactggtacgtcgatggcgtggaggtgcacaacgctaagaccaagcccagggaggagcagtacaattccacctacagggtggtgtccgtgctgaccgtcctccatcaggactggctgaacggcaaagagtataagtgcaaggtgagcaacaaggccctccctgctcccatcgagaagaccatcagcaaagccaagggccagcccagggaacctcaagtctataccctgcctcccagcagggaggagatgaccaagaaccaagtgagcctcacatgcctcgtcaagggcttctatccttccgatattgccgtcgagtgggagtccaacggacagcccgagaacaactacaagacaacaccccccgtgctcgattccgatggcagcttcttcctgtactccaagctgaccgtggacaagtccagatggcaacaaggcaacgtcttcagttgcagcgtcatgcatgaggccctccacaaccactacacccagaagagcctctccctgagccctggaaagtga

SEQ ID NO: 28 - DNA, 972 bp, synthetic construct
  source 1..972: mol_type = other DNA
gatattcagatgacccagagcccaagcagcctgtccgcatctgtcggagatagggtgactatcacctgcaaggcttccgaccacatcaacaattggctcgcctggtaccagcagaagcctggaaaggcccctaagttgctcatctccggcgccacatctcttgaaaccggggtgccaagtcggttttcagggagtggcagcgggactgactatacactgacaatttcctccctgcaacccgaggacttcgccacatactactgtcagcagtactggagcacaccctttactttcgggagcggcaccaaactggagattaagagaaccgtcgccgctcccagcgtcttcatcttcccccccagcgatgagcagctgaagagcggaaccgccagcgtggtgtgcctgctgaacaacttctaccccagggaggccaaggtgcaatggaaggtggacaacgccctacagagcggcaactcccaggagagcgtgaccgagcaggacagcaaggatagcacctacagcctgagcagcaccctcaccctgagcaaggccgactacgagaagcacaaggtgtacgcctgcgaggtgacccatcagggcctgagcagccctgtgaccaagagcttcaacaggggcgagtgcggcggaggcggaagcggaggaggaggatccgatactggaaggccatttgtggagatgtacagcgagatcccagagatcattcacatgacagaaggaagggagctcgtcatcccatgcagagtgacaagccctaacatcactgtcactctcaagaagttcccactcgacacactcatcccagatggcaagagaatcatttgggacagcagaaagggcttcatcatctccaacgccacatataaggagatcggactgctcacttgcgaagctacagtcaacggccacctctataagactaactatctgactcataggcaaacaaactgataa

SEQ ID NO: 29 - DNA, 1002 bp, synthetic construct
  source 1..1002: mol_type = other DNA
gatactggaaggccatttgtggagatgtacagcgagatcccagagatcattcacatgacagaaggaagggagctcgtcatcccatgcagagtgacaagccctaacatcactgtcactctcaagaagttcccactcgacacactcatcccagatggcaagagaatcatttgggacagcagaaagggcttcatcatctccaacgccacatataaggagatcggactgctcacttgcgaagctacagtcaacggccacctctataagactaactatctgactcataggcaaacaaacggtggaggcggttcaggcggaggtggcagcggcggtggcgggtcgggagggggtggctctgatattcagatgacccagagcccaagcagcctgtccgcatctgtcggagatagggtgactatcacctgcaaggcttccgaccacatcaacaattggctcgcctggtaccagcagaagcctggaaaggcccctaagttgctcatctccggcgccacatctcttgaaaccggggtgccaagtcggttttcagggagtggcagcgggactgactatacactgacaatttcctccctgcaacccgaggacttcgccacatactactgtcagcagtactggagcacaccctttactttcgggagcggcaccaaactggagattaagagaaccgtcgccgctcccagcgtcttcatcttcccccccagcgatgagcagctgaagagcggaaccgccagcgtggtgtgcctgctgaacaacttctaccccagggaggccaaggtgcaatggaaggtggacaacgccctacagagcggcaactcccaggagagcgtgaccgagcaggacagcaaggatagcacctacagcctgagcagcaccctcaccctgagcaaggccgactacgagaagcacaaggtgtacgcctgcgaggtgacccatcagggcctgagcagccctgtgaccaagagcttcaacaggggcgagtgctgataa

SEQ ID NO: 30 - DNA, 1665 bp, synthetic construct
  source 1..1665: mol_type = other DNA
gaggtgcagctcgtcgaatctggaggcggcctcgtgcagcctggggggtctcttagattgtcctgcgcagcttcaggattcactttctccagcttcgacatgagctgggggaggcaggctccagggaagaggctggagtgggtcgcctttatgtcctccggaggcagtacatactaccccgatagtgtgaaagggaggtttaccatcagccgcgacaacagcaagaacaccctgtacctgcagatgaatagcctgcgggccgaggatacagccgtctactactgtgcccggggcgagcggtacggctcctattggggccaagggacactggtgactgtgagctccgcgagcaccaagggaccttccgtgtttcccctcgcccccagctccaaaagcaccagcggcggaacagctgctctcggctgtctcgtcaaggattacttccccgagcccgtgaccgtgagctggaacagcggagccctgacaagcggcgtccacaccttccctgctgtcctacagtcctccggactgtacagcctgagcagcgtggtgacagtccctagcagctccctgggcacccagacatatatttgcaacgtgaatcacaagcccagcaacaccaaggtcgataagaaggtggagcctaagtcctgcgacaagacccacacatgtcccccctgtcccgctcctgaactgctgggaggcccttccgtgttcctgttcccccctaagcccaaggacaccctgatgatttccaggacacccgaggtgacctgtgtggtggtggacgtcagccacgaggaccccgaggtgaaattcaactggtacgtcgatggcgtggaggtgcacaacgctaagaccaagcccagggaggagcagtacaattccacctacagggtggtgtccgtgctgaccgtcctccatcaggactggctgaacggcaaagagtataagtgcaaggtgagcaacaaggccctccctgctcccatcgagaagaccatcagcaaagccaagggccagcccagggaacctcaagtctataccctgcctcccagcagggaggagatgaccaagaaccaagtgagcctcacatgcctcgtcaagggcttctatccttccgatattgccgtcgagtgggagtccaacggacagcccgagaacaactacaagacaacaccccccgtgctcgattccgatggcagcttcttcctgtactccaagctgaccgtggacaagtccagatggcaacaaggcaacgtcttcagttgcagcgtcatgcatgaggccctccacaaccactacacccagaagagcctctccctgagccctggagccggcggaggcggaagcggaggaggaggatccgatactggaaggccatttgtggaggcctacagcgagatcccagagatcattcacatgacagaaggaagggagctcgtcatcccatgcagagtgacaagccctaacatcactgtcactctcaagaagttcccactcgacacactcatcccagatggcaagagaatcatttgggacagcagaaagggcttcatcatctccaacgccacatataaggagatcggactgctcacttgcgaagctacagtcaacggccacctctataagactaactatctgactcataggcaaacaaactgataa

SEQ ID NO: 31 - DNA, 1665 bp, synthetic construct
  source 1..1665: mol_type = other DNA
gaggtgcagctcgtcgaatctggaggcggcctcgtgcagcctggggggtctcttagattgtcctgcgcagcttcaggattcactttctccagcttcgacatgagctgggggaggcaggctccagggaagaggctggagtgggtcgcctttatgtcctccggaggcagtacatactaccccgatagtgtgaaagggaggtttaccatcagccgcgacaacagcaagaacaccctgtacctgcagatgaatagcctgcgggccgaggatacagccgtctactactgtgcccggggcgagcggtacggctcctattggggccaagggacactggtgactgtgagctccgcgagcaccaagggaccttccgtgtttcccctcgcccccagctccaaaagcaccagcggcggaacagctgctctcggctgtctcgtcaaggattacttccccgagcccgtgaccgtgagctggaacagcggagccctgacaagcggcgtccacaccttccctgctgtcctacagtcctccggactgtacagcctgagcagcgtggtgacagtccctagcagctccctgggcacccagacatatatttgcaacgtgaatcacaagcccagcaacaccaaggtcgataagaaggtggagcctaagtcctgcgacaagacccacacatgtcccccctgtcccgctcctgaactgctgggaggcccttccgtgttcctgttcccccctaagcccaaggacaccctgatgatttccaggacacccgaggtgacctgtgtggtggtggacgtcagccacgaggaccccgaggtgaaattcaactggtacgtcgatggcgtggaggtgcacaacgctaagaccaagcccagggaggagcagtacaattccacctacagggtggtgtccgtgctgaccgtcctccatcaggactggctgaacggcaaagagtataagtgcaaggtgagcaacaaggccctccctgctcccatcgagaagaccatcagcaaagccaagggccagcccagggaacctcaagtctataccctgcctcccagcagggaggagatgaccaagaaccaagtgagcctcacatgcctcgtcaagggcttctatccttccgatattgccgtcgagtgggagtccaacggacagcccgagaacaactacaagacaacaccccccgtgctcgattccgatggcagcttcttcctgtactccaagctgaccgtggacaagtccagatggcaacaaggcaacgtcttcagttgcagcgtcatgcatgaggccctccacaaccactacacccagaagagcctctccctgagccctggagccggcggaggcggaagcggaggaggaggatccgatactggaaggccatttgtggagccctacagcgagatcccagagatcattcacatgacagaaggaagggagctcgtcatcccatgcagagtgacaagccctaacatcactgtcactctcaagaagttcccactcgacacactcatcccagatggcaagagaatcatttgggacagcagaaagggcttcatcatctccaacgccacatataaggagatcggactgctcacttgcgaagctacagtcaacggccacctctataagactaactatctgactcataggcaaacaaactgataa

SEQ ID NO: 32 - DNA, 1665 bp, synthetic construct
  source 1..1665: mol_type = other DNA
gaggtgcagctcgtcgaatctggaggcggcctcgtgcagcctggggggtctcttagattgtcctgcgcagcttcaggattcactttctccagcttcgacatgagctgggggaggcaggctccagggaagaggctggagtgggtcgcctttatgtcctccggaggcagtacatactaccccgatagtgtgaaagggaggtttaccatcagccgcgacaacagcaagaacaccctgtacctgcagatgaatagcctgcgggccgaggatacagccgtctactactgtgcccggggcgagcggtacggctcctattggggccaagggacactggtgactgtgagctccgcgagcaccaagggaccttccgtgtttcccctcgcccccagctccaaaagcaccagcggcggaacagctgctctcggctgtctcgtcaaggattacttccccgagcccgtgaccgtgagctggaacagcggagccctgacaagcggcgtccacaccttccctgctgtcctacagtcctccggactgtacagcctgagcagcgtggtgacagtccctagcagctccctgggcacccagacatatatttgcaacgtgaatcacaagcccagcaacaccaaggtcgataagaaggtggagcctaagtcctgcgacaagacccacacatgtcccccctgtcccgctcctgaactgctgggaggcccttccgtgttcctgttcccccctaagcccaaggacaccctgatgatttccaggacacccgaggtgacctgtgtggtggtggacgtcagccacgaggaccccgaggtgaaattcaactggtacgtcgatggcgtggaggtgcacaacgctaagaccaagcccagggaggagcagtacaattccacctacagggtggtgtccgtgctgaccgtcctccatcaggactggctgaacggcaaagagtataagtgcaaggtgagcaacaaggccctccctgctcccatcgagaagaccatcagcaaagccaagggccagcccagggaacctcaagtctataccctgcctcccagcagggaggagatgaccaagaaccaagtgagcctcacatgcctcgtcaagggcttctatccttccgatattgccgtcgagtgggagtccaacggacagcccgagaacaactacaagacaacaccccccgtgctcgattccgatggcagcttcttcctgtactccaagctgaccgtggacaagtccagatggcaacaaggcaacgtcttcagttgcagcgtcatgcatgaggccctccacaaccactacacccagaagagcctctccctgagccctggagccggcggaggcggaagcggaggaggaggatccgatactggaaggccatttgtggagacctacagcgagatcccagagatcattcacatgacagaaggaagggagctcgtcatcccatgcagagtgacaagccctaacatcactgtcactctcaagaagttcccactcgacacactcatcccagatggcaagagaatcatttgggacagcagaaagggcttcatcatctccaacgccacatataaggagatcggactgctcacttgcgaagctacagtcaacggccacctctataagactaactatctgactcataggcaaacaaactgataa

SEQ ID NO: 33 - DNA, 1665 bp, synthetic construct
  source 1..1665: mol_type = other DNA
gaggtgcagctcgtcgaatctggaggcggcctcgtgcagcctggggggtctcttagattgtcctgcgcagcttcaggattcactttctccagcttcgacatgagctgggggaggcaggctccagggaagaggctggagtgggtcgcctttatgtcctccggaggcagtacatactaccccgatagtgtgaaagggaggtttaccatcagccgcgacaacagcaagaacaccctgtacctgcagatgaatagcctgcgggccgaggatacagccgtctactactgtgcccggggcgagcggtacggctcctattggggccaagggacactggtgactgtgagctccgcgagcaccaagggaccttccgtgtttcccctcgcccccagctccaaaagcaccagcggcggaacagctgctctcggctgtctcgtcaaggattacttccccgagcccgtgaccgtgagctggaacagcggagccctgacaagcggcgtccacaccttccctgctgtcctacagtcctccggactgtacagcctgagcagcgtggtgacagtccctagcagctccctgggcacccagacatatatttgcaacgtgaatcacaagcccagcaacaccaaggtcgataagaaggtggagcctaagtcctgcgacaagacccacacatgtcccccctgtcccgctcctgaactgctgggaggcccttccgtgttcctgttcccccctaagcccaaggacaccctgatgatttccaggacacccgaggtgacctgtgtggtggtggacgtcagccacgaggaccccgaggtgaaattcaactggtacgtcgatggcgtggaggtgcacaacgctaagaccaagcccagggaggagcagtacaattccacctacagggtggtgtccgtgctgaccgtcctccatcaggactggctgaacggcaaagagtataagtgcaaggtgagcaacaaggccctccctgctcccatcgagaagaccatcagcaaagccaagggccagcccagggaacctcaagtctataccctgcctcccagcagggaggagatgaccaagaaccaagtgagcctcacatgcctcgtcaagggcttctatccttccgatattgccgtcgagtgggagtccaacggacagcccgagaacaactacaagacaacaccccccgtgctcgattccgatggcagcttcttcctgtactccaagctgaccgtggacaagtccagatggcaacaaggcaacgtcttcagttgcagcgtcatgcatgaggccctccacaaccactacacccagaagagcctctccctgagccctggagccggcggaggcggaagcggaggaggaggatccgatactggaaggccatttgtggaggccgccagcgagatcccagagatcattcacatgacagaaggaagggagctcgtcatcccatgcagagtgacaagccctaacatcactgtcactctcaagaagttcccactcgacacactcatcccagatggcaagagaatcatttgggacagcagaaagggcttcatcatctccaacgccacatataaggagatcggactgctcacttgcgaagctacagtcaacggccacctctataagactaactatctgactcataggcaaacaaactgataa

SEQ ID NO: 34 - protein, 98 aa, synthetic construct
DTGRPFVEMYSEIPEIIHMTEGRELVIPCRVTSPNITVTLKKFPLDTLIPDGKRIIWDSRKGFIISNATYKEIGLLTCEATVNGHLYKTNYLTHRQTN